European Patent Specification EP 3 665 301 B1, published October 4, 2023. Title: METHOD FOR PREDICTING THE RESPONSE OF NON-SMALL-CELL LUNG CARCINOMA PATIENTS TO A MEDICAMENT. Applicant: PamGene B.V. Erasmus University Medical Center Rotterdam. The sequence listing filed with the application follows.

SEQUENCE LISTING (22 sequences)

SEQ ID NO: 1 - protein, 12 aa, artificial sequence
  ART_004_EAIYAAPFAKKKXC
EAIYAAPFAKKK

SEQ ID NO: 2 - protein, 13 aa, artificial sequence
  ERBB4_1277_1289
IVAENPEYLSEFS

SEQ ID NO: 3 - protein, 13 aa, artificial sequence
  FGFR2_762_774
TLTTNEEYLDLSQ

SEQ ID NO: 4 - protein, 13 aa, artificial sequence
  LAT_194_206
MESIDDYVNVPES

SEQ ID NO: 5 - protein, 13 aa, artificial sequence
  ZAP70_485_497
ALGADDSYYTARS

SEQ ID NO: 6 - protein, 13 aa, artificial sequence
  MK01_180_192
HTGFLTEYVATRW

SEQ ID NO: 7 - protein, 13 aa, artificial sequence
  FAK2_572_584
RYIEDEDYYKASV

SEQ ID NO: 8 - protein, 13 aa, artificial sequence
  PAXI_24_36
FLSEETPYSYPTG

SEQ ID NO: 9 - protein, 13 aa, artificial sequence
  TNNT1_2_14
SDTEEQEYEEEQP

SEQ ID NO: 10 - protein, 13 aa, artificial sequence
  ANXA1_14_26
IENEEQEYVQTVK

SEQ ID NO: 11 - protein, 13 aa, artificial sequence
  DYR1A_212_224
KHDTEMKYYIVHL

SEQ ID NO: 12 - protein, 13 aa, artificial sequence
  41 _654_666
LDGENIYIRHSNL

SEQ ID NO: 13 - protein, 13 aa, artificial sequence
  FGFR3_753_765
TVTSTDEYLDLSA

SEQ ID NO: 14 - protein, 13 aa, artificial sequence
  LAT_249_261
EEGAPDYENLQEL

SEQ ID NO: 15 - protein, 13 aa, artificial sequence
  CBL_693_705
EGEEDTEYMTPSS

SEQ ID NO: 16 - protein, 13 aa, artificial sequence
  KSYK_518_530
ALRADENYYKAQT

SEQ ID NO: 17 - protein, 15 aa, artificial sequence
  PGFRB_1014_1028
PNEGDNDYIIPLPDP

SEQ ID NO: 18 - protein, 13 aa, artificial sequence
  EPOR_361_373
SEHAQDTYLVLDK

SEQ ID NO: 19 - protein, 13 aa, artificial sequence
  JAK1_1015_1027
AIETDKEYYTVKD

SEQ ID NO: 20 - protein, 13 aa, artificial sequence
  PRRX2_202_214
WTASSPYSTVPPY

SEQ ID NO: 21 - protein, 13 aa, artificial sequence
  PDPK1_369_381
DEDCYGNYDNLLS

SEQ ID NO: 22 - protein, 13 aa, artificial sequence
  EPHA1_774_786
LDDFDGTYETQGG